European Patent Specification EP 3 378 482 B1, published February 21, 2024. Title: Antitumor Drug Delivery Preparation. Applicant: Public University Corporation NAGOYA CITY UNIVERSITY THE UNIVERSITY OF TOKYO. The sequence listing filed with the application follows.

SEQUENCE LISTING (57 sequences)

SEQ ID NO: 1 - RNA, 7598 nt, Homo sapiens
uccugcuuuccugacccucuccgccauuuaaagaaacaguaccgggggcgggccgagcgacgcagccgggacgguagcugcggugcggaccggaggagccaucuugucucgucgccggggagucaggccccuaaaucgaagaagcccuggcgcgcccucccccccucccgggucugguagggcgaaggaacgggcgugcggucgaucgagcgaucgguuggcggcucuuucuccugcucuggcauccagcucuuggggcgcaggcccggccgccgcggcgcgcgcccgguggccguuggcgcucgcgccgcgucuuucuucucguacgcagaacucgggcggcggccuaugcguuugcgauucgacgaggagucguccggguggucggcggcggcgggcagcugcuccgccccgcuccgggggaggcggcggcggcagcggccgcgggauuuggagcggccggggaggcggggguggccggggccggcuuggaggccuggcgccacccuucggggccugcaaggacccaguugggggggcaggagggggccggaggaugguugguugugggauuucuacuuugccuuuuccuccuuaugccgccuuagugaggggcgggagcucuggcggcagccccgggguggggagacgagcuccggagucggaagagcuggguuuucuuccgggccuagccaccaguuggcggagugaccuuaggcgagucacucuguaauuugucugcgccucaguuuccuccucugccuaucaaugugugugggguugaaaucgcuuuguaaacuauaaagcguggguguacguaaaggaugguuauuguuuauaauuuuuuuugaguuguaagaaaacuuagcaguuccccaauccuuggguuuugaaccugggaaccuuggauuggaguuggggauccccaaacuuccugaaauugugggaaugugcgguuugggggaaugaugggaauuugugggaaugugcguuuuaggggaaugaugauccaucgcuagcaaguuuuccaagggggcugugacccagaagaguuaagaaucacaauuucuucaugcuacagagaggaaacugaggccuagaugucauuugggacccuucacaaccauuuugaagcccuguuugagucccugggauaugugagcuguuucuaugcauaauggauauucgggguuaacaacaguccccugcuuggcuucuauucugaauccuuuucuuucaccauggggugccugaaggguggcugaugcauaugguacaauggcacccaguguaaagcagcuacaauuaggaguggauguguucuguagcauccuauuuaaauaagccuauuuuauccuuuggcccgucaacucuguuaucugcugcuuguacuggugccuguacuuuucugacucucauugaccauauuccacgaccaugguugucauccauuacuugauccuacuuuacaugucuaggcugugugguugguggugaauaggcuucuuuuuacauggugcugccagcccagcuaauuaauggugcacguggacuuuuagcaagcgggcucacuggaagagacugaaccuggcauggaauuccugaagauguuugggguuuuuuucuuucuuaaucgaaaguuaacauugucugaaaaguuuuguuagaacuacugcggaaccucaaaaucaguagauuuggaagugauucaaagcuaaacuuuuuccuuggcccuccuuguguucuaauugcuugcaaguguaauacuaggauguccaagaugccaguuuuugcuucuuuguuaguugucagcugcuuuuaucaaauuucaggccauuauccaacaaacacuauaaaaauguuugaacaauuggauuucaaacauuuucguuuuguggaguggugcucaccaagugguacagcccuaagcaagugaacacaaacacauuuaaguguauuuugucugauuagauguuagccaguuaugcuauuucauucaaaugucugaaaaaaucaauugacuauucccuuuuccuaaagggcagagacagauaaucucacuuccagagaaaugacuuggagaaaaaaaaguguuggucuuuuugcucuuuuguaauuaaauccggauguaccucaaaagacuuaagacuguggugauaagaugcuuuccucagcagaaaggagggaaaaaaaacaacuggaacucaaagcuugaaauucuguggcaaaacaugagauguccaggauuggagguugaaaagauuucacuacaguguucugcaauaguuggagcagauaacuuucaguguagccacagccauggacuccagauuuccagauuuucaagaccuggaccuggaacccgaaagagcuugucacgaugcggcaggaacacuggagguagauuuuuuuuuauuuuugaauuuugggacuguugaccuugcugugagaaaagagacaacgacugagcaagcacuaccaccagcacuguuacugggaauuagaagaccugaguuucuguccagacccucagugcaaacugaggaugcuccauccaaagugaauuaugauagcagacuccuugaaagcaggguccuuguuuagugcaucuuugcccacauacaccacaacauaucaagaugcauuuauuaggaaggaggaguuuagagagcaggcuaucagaauaaccacucaccuacagaccugguaccuggauuuuugcccgagaugauuccuaccaccuuacuacugacgaagacacccauuccaguggaccacugugacccaggaggcauucagccaucaugauguggccuuuaccuccacuccugucuuguucuacccagauucagcacagcccuuuauagugaagucagaguccucaagccaaauagcuaaagcuguuuuaucacaacaaaggccuaguuuguuccaugagugugcauuucauuucuucaguuaaagccuucagagacacacaauaaauuuggaccaggggauuuuuuaguuauuaaugcucucugaagaaaggcaacaucuuuuugagagcagcauuggaccacaccccacaaucucaaaugauugaaauucaugaacaucuaggaucccgugaaggucacuggacccuguuuuuucuacuucaaauccuguaguagccuacugaaugagaaaacauauucugacccauugggaucaaaucaaaggcacagugaacuccucauagcaucuucuuuggaauuacucaggaaccagaacuuuuuacacaaauguaagaaauucuaccaaggaguccccuuaccuaacagcaucucacaaggcugcaccagauuccagaaaaggcuucucuugauacaucaagguagaaccucuaugcauuuugugaccgacuuauucuuagaucauugguuuuccaaaggcuuuguggccaugaagcccuuugagugaaaacugugcagaagcccagaguaaaagugaagcugcucuggaugaaguagugaagcaagaguaggggccugaauccugcuacaacuaucuuccuuuaccaccguggugacaccuaaggggacuuccuuacaacaccuugaacucuuccgaacacaguuugaaaaccacugccccagacagcaauauguuugaccugaauggcauuccaaucuuuucuguaccuccacucagcacaguucauguucaguagaugcugaacauucuuagaaauacugugugugaacuuagaaaagugcaagaagacaggcaugucuuugaccccaggaaugaucauuugcugaagauggugucaagugaaccuagauuaacagcccuccacuccagauggauauccagugauuccuagaaugggauauagccagagaacaauucuaugcacccuacacugacagacucccuuaagcaacaccagaugcucuacugguacuugaaguacaugacuuugaagucuugacccuccaugaauaccugaauuaucagcaagcggguuuugaagcuggugccucauugaggccauauuagagcaacuuguacauuugaccucuuguuaucagccaugguacucuacuucgugugcaagagauaacuaugaaagccaaauucaaauacuggcaacauuuccuaaaggggcucaauaucuaucauucgucuucuuuuccaaacuacacaucacuguaugacucaaccaguagcaguuauauugccccuugguuuuuauucaguuuaacuacuguuuccaagauaaaugagcuaauaagcuuuaaaaaaaaaaaaaaaaaaggcugaauucuuuuuucuucaucacuggcauaucugccuauucuccagaauuauuaugacuauucagcucacuuuaacaguugaacuucaagcgacaaucuuugaacaccccuucucaugugauuuaaaaugaaaccauuuggaaaaguuucuucuagccaguaauagauuuuuuuuuuaauugcucugccuugugccgagagauguucuuuuaagaugaaucuuuugaugucugauaccaccaaauauaggugguagggagaguuggaggcuggcccuuugagcaggccauuagcuuacuugcugggcauuuccgauagcuuauugccuaccuuuuugcuggaaacaaacugauuugaaaaacaaaaucuaugaagacugcagcuaaggauuuuaucgguagacuuaagagcuuuuguccuuguggauauuuuaguggaaccacaucagucucaauacugucauuuuacacugacucagagcagcugacuucauuccuugccaugauauauauuuaaggcaggcauuguaacagacauaaagacaacuuaucuguuucagcaggaaggauucaguuuaugaacucucagaccagaucauguugaacaaggagacuuugaugugugucaugagaaaacucauucuuuacuucccagucaauuuaaaggccagcuauccugagcuacucgaaugaaugcacugguuaaacauuggaaauaguuuguuuauauccuugucucucucuaggccaauugugauuacaugacucgacucuacaucucgucaaacaaggccuaggucugguugcuguagacugcucgcccucaacaaauaaaaucugguugacuagccuccuuguauauacaacuauuauuuguuaagaagaaauuaucgucaauuuucuacuaccuuccaauugucagcucuuuuuuuccucucugguuuuuccuauacuuuacagaaaaagacauugaucuauacugccauucccucuaauccugccauacucagucaaaaggaaugacuuaagaugaagaugaucaucugcucgagucuaaaauauacauuguauauaagaauuggugauuagaaaagcaaaaaaccuaaaacuuaaaucuaggagucuguauacugucuccaugucuccaugccucagaucucaucuaaaucuuugaacagcaccauucaaccaaucugaggccuugacuugcuuguaagaugauucucagagaucggcugaguuaaaaaagaugacgacuugauuaccaaagaaaguagggccaacuuugacaaaucuggcucugcugacccugucacucccagauguagcauagacuccuaaacagaaccucaagucugauugaggauaaggccuucuccugagcugaaaguucuuuggcagaugagcaagaaacugaaagcugauguaccugacuggcucuguaagaucagaaaacuguauccagaauaagcccuauggauuaaccccugaguacccagaguaaaaacuaauuuacagaacuuccuuauugaucugcugguucuuccagaucauauucuggcuauugguauggcuggccuuucugaagguacccugcuugucuauuuuccugacucagcucuugccugccuuuuucacauguugcugcaauuagacucaccgugaggacuacagucaauuucagucuaucuugugcccaauacaacaaggauuuuuaauaguaacaacccacaccucacccacuaggacucaauguucacaacaggaaggaccauugcugcauacuccuugaccagcaacuuuuuugaagauauuuuuaagugcagaguaggccucuauuccuguauguaauuguucauuuucagcaccuggaaccucaucuaucgggucuggaaggaauacagcaguucgaaagccgcguccauuucucuccuucaguagugcagaaaugaguccgauucaccaguacacacagaacuguaccaguucaaccuagcaaaagaagaaaaguuuccacuguacuuaaaauuuacagcugacucaaauugccucacagaauuauuugauguagaaggcuaguugucuuacuucagaucagcaggacaguugggcucucagacucaugaccacugaguuugcuuguguugaaacugugguuucauccaacauaugcuauuggacaugauuauuauuccauucaaauggauuacagacuucuugaggacaggacaaacuuaucucucaugguguuuuuuuagaauacuuuuauaaccaaggaagaaaccaugccagcuguuaccauucaacuucuuaagcagagauuaagcuuuuucauaucuguucuuauccuggacaucaguaguuuuuaauugcccagcauccguuccaucuuguaacaacucccugauguuucuuaaaaccaccucuuccuauuuucagucugugguuuggacagucugacccaaccuugagcuuugugggugaacauguaauucagaccucaucaaucagcaaauccaucugaacuguggaggagaagcucucuuuacugagggugcuuuagcuuuguaggaugaaaaccucaaacuaacagggccuaccauguagagaaugaagccagugcaggggaaagcagagccaaaauauggagagacuugaauccugaugacagcguuugugccccuggauccaaccgugccugaagcuagaauauccccuggacuuuucaguuaugugaaccaauaaauacccuuuuuugcuuaaguuacuuugaguuggguuucuguuacuugaaauugaauccacacuaauauaucuaccaacauugagacuugacagauccaaguauuuauuaagcuagaggucauggucacugaaauuacuuuccaaaguggaagacaaaaugaaacaggaacugagggaauauuuaagaucccacagaagcguaaaaaugacaugguagaaaguaauagaaaaccuaaaugucugucauuaaaggauagguuaaggugugguucagccauauaggaauaucucguaucuguuaaaaugaauaaaguacauucauuguguauggaaaaauggccaugauacauuaggugaaacaaguuauuaauagaaaaguguacagugugaacucauuuuaaaaugugugugcuuauguuuauaaaugcauagaaaggucuauucacagcuuucuuugaacaguguagaucacaugaaacuuucaacuuuauacauuucuguauuaauauuuuacacuacccacauuauuuuuaaacuuuauuuuaaauaaagaauuuuuaaaauuaaa

SEQ ID NO: 2 - RNA, 7528 nt, Homo sapiens
uccugcuuuccugacccucuccgccauuuaaagaaacaguaccgggggcgggccgagcgacgcagccgggacgguagcugcggugcggaccggaggagccaucuugucucgucgccggggagucaggccccuaaaucgaagaagcccuggcgcgcccucccccccucccgggucugguagggcgaaggaacgggcgugcggucgaucgagcgaucgguuggcggcucuuucuccugcucuggcauccagcucuuggggcgcaggcccggccgccgcggcgcgcgcccgguggccguuggcgcucgcgccgcgucuuucuucucguacgcagaacucgggcggcggccuaugcguuugcgauucgacgaggagucguccggguggucggcggcggcgggcagcugcuccgccccgcuccgggggaggcggcggcggcagcggccgcgggauuuggagcggccggggaggcggggguggccggggccggcuuggaggccuggcgccacccuucggggccugcaaggacccaguugggggggcaggagggggccggaggaugguugguugugggauuucuacuuugccuuuuccuccuuaugccgccuuagugaggggcgggagcucuggcggcagccccgggguggggagacgagcuccggagucggaagagcuggguuuucuuccgggccuagccaccaguuggcggagugaccuuaggcgagucacucuguaauuugucugcgccucaguuuccuccucugccuaucaaugugugugggguugaaaucgcuuuguaaacuauaaagcguggguguacguaaaggaugguuauuguuuauaauuuuuuuugaguuguaagaaaacuuagcaguuccccaauccuuggguuuugaaccugggaaccuuggauuggaguuggggauccccaaacuuccugaaauugugggaaugugcgguuugggggaaugaugggaauuugugggaaugugcguuuuaggggaaugaugauccaucgcuagcaaguuuuccaagggggcugugacccagaagaguuaagaaucacaauuucuucaugcuacagagaggaaacugaggccuagaugucauuugggacccuucacaaccauuuugaagcccuguuugagucccugggauaugugagcuguuucuaugcauaauggauauucgggguuaacaacaguccccugcuuggcuucuauucugaauccuuuucuuucaccauggggugccugaaggguggcugaugcauaugguacaauggcacccaguguaaagcagcuacaauuaggaguggauguguucuguagcauccuauuuaaauaagccuauuuuauccuuuggcccgucaacucuguuaucugcugcuuguacuggugccuguacuuuucugacucucauugaccauauuccacgaccaugguugucauccauuacuugauccuacuuuacaugucuaggcugugugguugguggugaauaggcuucuuuuuacauggugcugccagcccagcuaauuaauggugcacguggacuuuuagcaagcgggcucacuggaagagacugaaccuggcauggaauuccugaagauguuugggguuuuuuucuuucuuaaucgaaaguuaacauugucugaaaaguuuuguuagaacuacugcggaaccucaaaaucaguagauuuggaagugauucaaagcuaaacuuuuuccuuggcccuccuuguguucuaauugcuugcaaguguaauacuaggauguccaagaugccaguuuuugcuucuuuguuaguugucagcugcuuuuaucaaauuucaggccauuauccaacaaacacuauaaaaauguuugaacaauuggauuucaaacauuuucguuuuguggaguggugcucaccaagugguacagcccuaagcaagugaacacaaacacauuuaaguguauuuugucugauuagauguuagccaguuaugcuauuucauucaaaugucugaaaaaaucaauugacuauucccuuuuccuaaagggcagagacagauaaucucacuuccagagaaaugacuuggagaaaaaaaaguguuggucuuuuugcucuuuuguaauuaaauccggauguaccucaaaagacuuaagacuguggugauaagaugcuuuccucagcagaaaggagggaaaaaaaacaacuggaacucaaagcuugaaauucuguggcaaaacaugagauguccaggauuggagguugaaaagauuucacuacaguguucugcaauaguuggagcagauaacuuucaguguagccacagccauggacuccagauuuccagauuuucaagaccuggaccuggaacccgaaagagcuugucacgaugcggcaggaacacuggagguagauuuuuuuuuauuuuugaauuuugggacuguugaccuugcugugagaaaagagacaacgacugagcaagcacuaccaccagcacuguuacugggaauuagaagaccugaguuucuguccagacccucagugcaaacugaggaugcuccauccaaagugaauuauguccugugccuccugauugcugaguguucaccuggaccuucugacuaccuucccugugcuauuccaucagccuacagaccugguaccuggauuuuugcccgagaugauuccuaccaccuuacuacugacgaagacacccauuccaguggaccacugugacccaggaggcauucagccaucaugauguggccuuuaccuccacuccugucuuguucuacccagauucagcacagcccuuuauagugaagucagaguccucaagccaaauagcuaaagcuguuuuaucacaacaaaggccuaguuuguuccaugagugugcauuucauuucuucaguuaaagccuucagagacacacaauaaauuuggaccaggggauuuuuuaguuauuaaugcucucugaagaaaggcaacaucuuuuugagagcagcauuggaccacaccccacaaucucaaaugauugaaauucaugaacaucuaggaucccgugaaggucacuggacccuguuuuuucuacuucaaauccuguaguagccuacugaaugagaaaacauauucugacccauugggaucaaaucaaaggcacagugaacuccucauagcaucuucuuuggaauuacucaggaaccagaacuuuuuacacaaauguaagaaauucuaccaaggaguccccuuaccuaacagcaucucacaaggcugcaccagauuccagaaaaggcuucucuugauacaucaagcauuuugugaccgacuuauucuuagaucauugguuuuccaaaggcuuuguggccaugaagcccuuugagugaaaacugugcagaagcccagaguaaaagugaagcugcucuggaugaaguagugaagcaagaguaggggccugaauccugcuacaacuaucuuccuuuaccaccguggugacaccuaaggggacuuccuuacaacaccuugaacucuuccgaacacaguuugaaaaccacugccccagacagcaauauguuugaccugaauggcauuccaaucuuuucuguaccuccacucagcacaguucauguucaguagaugcugaacauucuuagaaauacugugugugaacuuagaaaagugcaagaagacaggcaugucuuugaccccaggaaugaucauuugcugaagauggugucaagugaaccuagauuaacagcccuccacuccagauggauauccagugauuccuagaaugggauauagccagagaacaauucuaugcacccuacacugacagacucccuuaagcaacaccagaugcucuacugguacuugaaguacaugacuuugaagucuugacccuccaugaauaccugaauuaucagcaagcggguuuugaagcuggugccucauugaggccauauuagagcaacuuguacauuugaccucuuguuaucagccaugguacucuacuucgugugcaagagauaacuaugaaagccaaauucaaauacuggcaacauuuccuaaaggggcucaauaucuaucauucgucuucuuuuccaaacuacacaucacuguaugacucaaccaguagcaguuauauugccccuugguuuuuauucaguuuaacuacuguuuccaagauaaaugagcuaauaagcuuuaaaaaaaaaaaaaaaaaaggcugaauucuuuuuucuucaucacuggcauaucugccuauucuccagaauuauuaugacuauucagcucacuuuaacaguugaacuucaagcgacaaucuuugaacaccccuucucaugugauuuaaaaugaaaccauuuggaaaaguuucuucuagccaguaauagauuuuuuuuuuaauugcucugccuugugccgagagauguucuuuuaagaugaaucuuuugaugucugauaccaccaaauauaggugguagggagaguuggaggcuggcccuuugagcaggccauuagcuuacuugcugggcauuuccgauagcuuauugccuaccuuuuugcuggaaacaaacugauuugaaaaacaaaaucuaugaagacugcagcuaaggauuuuaucgguagacuuaagagcuuuuguccuuguggauauuuuaguggaaccacaucagucucaauacugucauuuuacacugacucagagcagcugacuucauuccuugccaugauauauauuuaaggcaggcauuguaacagacauaaagacaacuuaucuguuucagcaggaaggauucaguuuaugaacucucagaccagaucauguugaacaaggagacuuugaugugugucaugagaaaacucauucuuuacuucccagucaauuuaaaggccagcuauccugagcuacucgaaugaaugcacugguuaaacauuggaaauaguuuguuuauauccuugucucucucuaggccaauugugauuacaugacucgacucuacaucucgucaaacaaggccuaggucugguugcuguagacugcucgcccucaacaaauaaaaucugguugacuagccuccuuguauauacaacuauuauuuguuaagaagaaauuaucgucaauuuucuacuaccuuccaauugucagcucuuuuuuuccucucugguuuuuccuauacuuuacagaaaaagacauugaucuauacugccauucccucuaauccugccauacucagucaaaaggaaugacuuaagaugaagaugaucaucugcucgagucuaaaauauacauuguauauaagaauuggugauuagaaaagcaaaaaaccuaaaacuuaaaucuaggagucuguauacugucuccaugucuccaugccucagaucucaucuaaaucuuugaacagcaccauucaaccaaucugaggccuugacuugcuuguaagaugauucucagagaucggcugaguuaaaaaagaugacgacuugauuaccaaagaaaguagggccaacuuugacaaaucuggcucugcugacccugucacucccagauguagcauagacuccuaaacagaaccucaagucugauugaggauaaggccuucuccugagcugaaaguucuuuggcagaugagcaagaaacugaaagcugauguaccugacuggcucuguaagaucagaaaacuguauccagaauaagcccuauggauuaaccccugaguacccagaguaaaaacuaauuuacagaacuuccuuauugaucugcugguucuuccagaucauauucuggcuauugguauggcuggccuuucugaagguacccugcuugucuauuuuccugacucagcucuugccugccuuuuucacauguugcugcaauuagacucaccgugaggacuacagucaauuucagucuaucuugugcccaauacaacaaggauuuuuaauaguaacaacccacaccucacccacuaggacucaauguucacaacaggaaggaccauugcugcauacuccuugaccagcaacuuuuuugaagauauuuuuaagugcagaguaggccucuauuccuguauguaauuguucauuuucagcaccuggaaccucaucuaucgggucuggaaggaauacagcaguucgaaagccgcguccauuucucuccuucaguagugcagaaaugaguccgauucaccaguacacacagaacuguaccaguucaaccuagcaaaagaagaaaaguuuccacuguacuuaaaauuuacagcugacucaaauugccucacagaauuauuugauguagaaggcuaguugucuuacuucagaucagcaggacaguugggcucucagacucaugaccacugaguuugcuuguguugaaacugugguuucauccaacauaugcuauuggacaugauuauuauuccauucaaauggauuacagacuucuugaggacaggacaaacuuaucucucaugguguuuuuuuagaauacuuuuauaaccaaggaagaaaccaugccagcuguuaccauucaacuucuuaagcagagauuaagcuuuuucauaucuguucuuauccuggacaucaguaguuuuuaauugcccagcauccguuccaucuuguaacaacucccugauguuucuuaaaaccaccucuuccuauuuucagucugugguuuggacagucugacccaaccuugagcuuugugggugaacauguaauucagaccucaucaaucagcaaauccaucugaacuguggaggagaagcucucuuuacugagggugcuuuagcuuuguaggaugaaaaccucaaacuaacagggccuaccauguagagaaugaagccagugcaggggaaagcagagccaaaauauggagagacuugaauccugaugacagcguuugugccccuggauccaaccgugccugaagcuagaauauccccuggacuuuucaguuaugugaaccaauaaauacccuuuuuugcuuaaguuacuuugaguuggguuucuguuacuugaaauugaauccacacuaauauaucuaccaacauugagacuugacagauccaaguauuuauuaagcuagaggucauggucacugaaauuacuuuccaaaguggaagacaaaaugaaacaggaacugagggaauauuuaagaucccacagaagcguaaaaaugacaugguagaaaguaauagaaaaccuaaaugucugucauuaaaggauagguuaaggugugguucagccauauaggaauaucucguaucuguuaaaaugaauaaaguacauucauuguguauggaaaaauggccaugauacauuaggugaaacaaguuauuaauagaaaaguguacagugugaacucauuuuaaaaugugugugcuuauguuuauaaaugcauagaaaggucuauucacagcuuucuuugaacaguguagaucacaugaaacuuucaacuuuauacauuucuguauuaauauuuuacacuacccacauuauuuuuaaacuuuauuuuaaauaaagaauuuuuaaaauuaaa

SEQ ID NO: 3 - RNA, 7542 nt, Homo sapiens
uccugcuuuccugacccucuccgccauuuaaagaaacaguaccgggggcgggccgagcgacgcagccgggacgguagcugcggugcggaccggaggagccaucuugucucgucgccggggagucaggccccuaaaucgaagaagcccuggcgcgcccucccccccucccgggucugguagggcgaaggaacgggcgugcggucgaucgagcgaucgguuggcggcucuuucuccugcucuggcauccagcucuuggggcgcaggcccggccgccgcggcgcgcgcccgguggccguuggcgcucgcgccgcgucuuucuucucguacgcagaacucgggcggcggccuaugcguuugcgauucgacgaggagucguccggguggucggcggcggcgggcagcugcuccgccccgcuccgggggaggcggcggcggcagcggccgcgggauuuggagcggccggggaggcggggguggccggggccggcuuggaggccuggcgccacccuucggggccugcaaggacccaguugggggggcaggagggggccggaggaugguugguugugggauuucuacuuugccuuuuccuccuuaugccgccuuagugaggggcgggagcucuggcggcagccccgggguggggagacgagcuccggagucggaagagcuggguuuucuuccgggccuagccaccaguuggcggagugaccuuaggcgagucacucuguaauuugucugcgccucaguuuccuccucugccuaucaaugugugugggguugaaaucgcuuuguaaacuauaaagcguggguguacguaaaggaugguuauuguuuauaauuuuuuuugaguuguaagaaaacuuagcaguuccccaauccuuggguuuugaaccugggaaccuuggauuggaguuggggauccccaaacuuccugaaauugugggaaugugcgguuugggggaaugaugggaauuugugggaaugugcguuuuaggggaaugaugauccaucgcuagcaaguuuuccaagggggcugugacccagaagaguuaagaaucacaauuucuucaugcuacagagaggaaacugaggccuagaugucauuugggacccuucacaaccauuuugaagcccuguuugagucccugggauaugugagcuguuucuaugcauaauggauauucgggguuaacaacaguccccugcuuggcuucuauucugaauccuuuucuuucaccauggggugccugaaggguggcugaugcauaugguacaauggcacccaguguaaagcagcuacaauuaggaguggauguguucuguagcauccuauuuaaauaagccuauuuuauccuuuggcccgucaacucuguuaucugcugcuuguacuggugccuguacuuuucugacucucauugaccauauuccacgaccaugguugucauccauuacuugauccuacuuuacaugucuaggcugugugguugguggugaauaggcuucuuuuuacauggugcugccagcccagcuaauuaauggugcacguggacuuuuagcaagcgggcucacuggaagagacugaaccuggcauggaauuccugaagauguuugggguuuuuuucuuucuuaaucgaaaguuaacauugucugaaaaguuuuguuagaacuacugcggaaccucaaaaucaguagauuuggaagugauucaaagcuaaacuuuuuccuuggcccuccuuguguucuaauugcuugcaaguguaauacuaggauguccaagaugccaguuuuugcuucuuuguuaguugucagcugcuuuuaucaaauuucaggccauuauccaacaaacacuauaaaaauguuugaacaauuggauuucaaacauuuucguuuuguggaguggugcucaccaagugguacagcccuaagcaagugaacacaaacacauuuaaguguauuuugucugauuagauguuagccaguuaugcuauuucauucaaaugucugaaaaaaucaauugacuauucccuuuuccuaaagggcagagacagauaaucucacuuccagagaaaugacuuggagaaaaaaaaguguuggucuuuuugcucuuuuguaauuaaauccggauguaccucaaaagacuuaagacuguggugauaagaugcuuuccucagcagaaaggagggaaaaaaaacaacuggaacucaaagcuugaaauucuguggcaaaacaugagauguccaggauuggagguugaaaagauuucacuacaguguucugcaauaguuggagcagauaacuuucaguguagccacagccauggacuccagauuuccagauuuucaagaccuggaccuggaacccgaaagagcuugucacgaugcggcaggaacacuggagguagauuuuuuuuuauuuuugaauuuugggacuguugaccuugcugugagaaaagagacaacgacugagcaagcacuaccaccagcacuguuacugggaauuagaagaccugaguuucuguccagacccucagugcaaacugaggaugcuccauccaaagugaauuauguccugugccuccugauugcugaguguucaccuggaccuucugacuaccuucccugugcuauuccaucagccuacagaccugguaccuggauuuuugcccgagaugauuccuaccaccuuacuacugacgaagacacccauuccaguggaccacugugacccaggaggcauucagccaucaugauguggccuuuaccuccacuccugucuuguucuacccagauucagcacagcccuuuauagugaagucagaguccucaagccaaauagcuaaagcuguuuuaucacaacaaaggccuaguuuguuccaugagugugcauuucauuucuucaguuaaagccuucagagacacacaauaaauuuggaccaggggauuuuuuaguuauuaaugcucucugaagaaaggcaacaucuuuuugagagcagcauuggaccacaccccacaaucucaaaugauugaaauucaugaacaucuaggaucccgugaaggucacuggacccuguuuuuucuacuucaaauccuguaguagccuacugaaugagaaaacauauucugacccauugggaucaaaucaaaggcacagugaacuccucauagcaucuucuuuggaauuacucaggaaccagaacuuuuuacacaaauguaagaaauucuaccaaggaguccccuuaccuaacagcaucucacaaggcugcaccagauuccagaaaaggcuucucuugauacaucaagguagaaccucuaugcauuuugugaccgacuuauucuuagaucauugguuuuccaaaggcuuuguggccaugaagcccuuugagugaaaacugugcagaagcccagaguaaaagugaagcugcucuggaugaaguagugaagcaagaguaggggccugaauccugcuacaacuaucuuccuuuaccaccguggugacaccuaaggggacuuccuuacaacaccuugaacucuuccgaacacaguuugaaaaccacugccccagacagcaauauguuugaccugaauggcauuccaaucuuuucuguaccuccacucagcacaguucauguucaguagaugcugaacauucuuagaaauacugugugugaacuuagaaaagugcaagaagacaggcaugucuuugaccccaggaaugaucauuugcugaagauggugucaagugaaccuagauuaacagcccuccacuccagauggauauccagugauuccuagaaugggauauagccagagaacaauucuaugcacccuacacugacagacucccuuaagcaacaccagaugcucuacugguacuugaaguacaugacuuugaagucuugacccuccaugaauaccugaauuaucagcaagcggguuuugaagcuggugccucauugaggccauauuagagcaacuuguacauuugaccucuuguuaucagccaugguacucuacuucgugugcaagagauaacuaugaaagccaaauucaaauacuggcaacauuuccuaaaggggcucaauaucuaucauucgucuucuuuuccaaacuacacaucacuguaugacucaaccaguagcaguuauauugccccuugguuuuuauucaguuuaacuacuguuuccaagauaaaugagcuaauaagcuuuaaaaaaaaaaaaaaaaaaggcugaauucuuuuuucuucaucacuggcauaucugccuauucuccagaauuauuaugacuauucagcucacuuuaacaguugaacuucaagcgacaaucuuugaacaccccuucucaugugauuuaaaaugaaaccauuuggaaaaguuucuucuagccaguaauagauuuuuuuuuuaauugcucugccuugugccgagagauguucuuuuaagaugaaucuuuugaugucugauaccaccaaauauaggugguagggagaguuggaggcuggcccuuugagcaggccauuagcuuacuugcugggcauuuccgauagcuuauugccuaccuuuuugcuggaaacaaacugauuugaaaaacaaaaucuaugaagacugcagcuaaggauuuuaucgguagacuuaagagcuuuuguccuuguggauauuuuaguggaaccacaucagucucaauacugucauuuuacacugacucagagcagcugacuucauuccuugccaugauauauauuuaaggcaggcauuguaacagacauaaagacaacuuaucuguuucagcaggaaggauucaguuuaugaacucucagaccagaucauguugaacaaggagacuuugaugugugucaugagaaaacucauucuuuacuucccagucaauuuaaaggccagcuauccugagcuacucgaaugaaugcacugguuaaacauuggaaauaguuuguuuauauccuugucucucucuaggccaauugugauuacaugacucgacucuacaucucgucaaacaaggccuaggucugguugcuguagacugcucgcccucaacaaauaaaaucugguugacuagccuccuuguauauacaacuauuauuuguuaagaagaaauuaucgucaauuuucuacuaccuuccaauugucagcucuuuuuuuccucucugguuuuuccuauacuuuacagaaaaagacauugaucuauacugccauucccucuaauccugccauacucagucaaaaggaaugacuuaagaugaagaugaucaucugcucgagucuaaaauauacauuguauauaagaauuggugauuagaaaagcaaaaaaccuaaaacuuaaaucuaggagucuguauacugucuccaugucuccaugccucagaucucaucuaaaucuuugaacagcaccauucaaccaaucugaggccuugacuugcuuguaagaugauucucagagaucggcugaguuaaaaaagaugacgacuugauuaccaaagaaaguagggccaacuuugacaaaucuggcucugcugacccugucacucccagauguagcauagacuccuaaacagaaccucaagucugauugaggauaaggccuucuccugagcugaaaguucuuuggcagaugagcaagaaacugaaagcugauguaccugacuggcucuguaagaucagaaaacuguauccagaauaagcccuauggauuaaccccugaguacccagaguaaaaacuaauuuacagaacuuccuuauugaucugcugguucuuccagaucauauucuggcuauugguauggcuggccuuucugaagguacccugcuugucuauuuuccugacucagcucuugccugccuuuuucacauguugcugcaauuagacucaccgugaggacuacagucaauuucagucuaucuugugcccaauacaacaaggauuuuuaauaguaacaacccacaccucacccacuaggacucaauguucacaacaggaaggaccauugcugcauacuccuugaccagcaacuuuuuugaagauauuuuuaagugcagaguaggccucuauuccuguauguaauuguucauuuucagcaccuggaaccucaucuaucgggucuggaaggaauacagcaguucgaaagccgcguccauuucucuccuucaguagugcagaaaugaguccgauucaccaguacacacagaacuguaccaguucaaccuagcaaaagaagaaaaguuuccacuguacuuaaaauuuacagcugacucaaauugccucacagaauuauuugauguagaaggcuaguugucuuacuucagaucagcaggacaguugggcucucagacucaugaccacugaguuugcuuguguugaaacugugguuucauccaacauaugcuauuggacaugauuauuauuccauucaaauggauuacagacuucuugaggacaggacaaacuuaucucucaugguguuuuuuuagaauacuuuuauaaccaaggaagaaaccaugccagcuguuaccauucaacuucuuaagcagagauuaagcuuuuucauaucuguucuuauccuggacaucaguaguuuuuaauugcccagcauccguuccaucuuguaacaacucccugauguuucuuaaaaccaccucuuccuauuuucagucugugguuuggacagucugacccaaccuugagcuuugugggugaacauguaauucagaccucaucaaucagcaaauccaucugaacuguggaggagaagcucucuuuacugagggugcuuuagcuuuguaggaugaaaaccucaaacuaacagggccuaccauguagagaaugaagccagugcaggggaaagcagagccaaaauauggagagacuugaauccugaugacagcguuugugccccuggauccaaccgugccugaagcuagaauauccccuggacuuuucaguuaugugaaccaauaaauacccuuuuuugcuuaaguuacuuugaguuggguuucuguuacuugaaauugaauccacacuaauauaucuaccaacauugagacuugacagauccaaguauuuauuaagcuagaggucauggucacugaaauuacuuuccaaaguggaagacaaaaugaaacaggaacugagggaauauuuaagaucccacagaagcguaaaaaugacaugguagaaaguaauagaaaaccuaaaugucugucauuaaaggauagguuaaggugugguucagccauauaggaauaucucguaucuguuaaaaugaauaaaguacauucauuguguauggaaaaauggccaugauacauuaggugaaacaaguuauuaauagaaaaguguacagugugaacucauuuuaaaaugugugugcuuauguuuauaaaugcauagaaaggucuauucacagcuuucuuugaacaguguagaucacaugaaacuuucaacuuuauacauuucuguauuaauauuuuacacuacccacauuauuuuuaaacuuuauuuuaaauaaagaauuuuuaaaauuaaa

SEQ ID NO: 4 - RNA, 19 nt, Artificial
  siRNA for human TUG1
ccagaagaguuaagaauca

SEQ ID NO: 5 - RNA, 19 nt, Artificial
  siRNA for human TUG1
gugcagaagcccagaguaa

SEQ ID NO: 6 - RNA, 21 nt, Artificial
  siRNA for human TUG1
ggauauagccagagaacaauu

SEQ ID NO: 7 - RNA, 21 nt, Artificial
  siRNA for human TUG1
guuaagaagaaauuaucguca

SEQ ID NO: 8 - RNA, 21 nt, Artificial
  siRNA for human TUG1
ggauuuuuuaguuauuaaugc

SEQ ID NO: 9 - RNA, 21 nt, Artificial
  siRNA for human TUG1
cucaaaugauugaaauucaug

SEQ ID NO: 10 - RNA, 21 nt, Artificial
  siRNA for human TUG1
ccuguuuuuucuacuucaaau

SEQ ID NO: 11 - RNA, 21 nt, Artificial
  siRNA for human TUG1
cacaaauguaagaaauucuac

SEQ ID NO: 12 - RNA, 19 nt, Artificial
  siRNA for human TUG1
ugauucuuaacucuucugg

SEQ ID NO: 13 - RNA, 19 nt, Artificial
  siRNA for human TUG1
uuacucugggcuucugcac

SEQ ID NO: 14 - RNA, 21 nt, Artificial
  siRNA for human TUG1
uuguucucuggcuauauccca

SEQ ID NO: 15 - RNA, 21 nt, Artificial
  siRNA for human TUG1
acgauaauuucuucuuaacaa

SEQ ID NO: 16 - RNA, 21 nt, Artificial
  siRNA for human TUG1
auuaauaacuaaaaaaucccc

SEQ ID NO: 17 - RNA, 21 nt, Artificial
  siRNA for human TUG1
ugaauuucaaucauuugagau

SEQ ID NO: 18 - RNA, 21 nt, Artificial
  siRNA for human TUG1
uugaaguagaaaaaacagggu

SEQ ID NO: 19 - RNA, 21 nt, Artificial
  siRNA for human TUG1
agaauuucuuacauuugugua

SEQ ID NO: 20 - DNA, 19 bp, Artificial
  siRNA for human TUG1
  misc_RNA (1)..(17)
ccagaagaguuaagaauca

SEQ ID NO: 21 - DNA, 19 bp, Artificial
  siRNA for human TUG1
  misc_RNA (1)..(17)
gugcagaagcccagaguaa

SEQ ID NO: 22 - DNA, 21 bp, Artificial
  siRNA for human TUG1
  misc_RNA (1)..(19)
ggauauagccagagaacaatt

SEQ ID NO: 23 - DNA, 21 bp, Artificial
  siRNA for human TUG1
  misc_RNA (1)..(19)
guuaagaagaaauuaucguca

SEQ ID NO: 24 - DNA, 21 bp, Artificial
  siRNA for human TUG1
  misc_RNA (1)..(19)
ggauuuuuuaguuauuaaugc

SEQ ID NO: 25 - DNA, 21 bp, Artificial
  siRNA for human TUG1
  misc_RNA (1)..(19)
cucaaaugauugaaauucatg

SEQ ID NO: 26 - DNA, 21 bp, Artificial
  siRNA for human TUG1
  misc_RNA (1)..(19)
ccuguuuuuucuacuucaaat

SEQ ID NO: 27 - DNA, 21 bp, Artificial
  siRNA for human TUG1
  misc_RNA (1)..(19)
cacaaauguaagaaauucuac

SEQ ID NO: 28 - DNA, 19 bp, Artificial
  siRNA for human TUG1
  misc_RNA (1)..(17)
ugauucuuaacucuucugg

SEQ ID NO: 29 - DNA, 19 bp, Artificial
  siRNA for human TUG1
  misc_RNA (1)..(17)
uuacucugggcuucugcac

SEQ ID NO: 30 - DNA, 21 bp, Artificial
  siRNA for human TUG1
  misc_RNA (1)..(19)
uuguucucuggcuauauccca

SEQ ID NO: 31 - DNA, 21 bp, Artificial
  siRNA for human TUG1
  misc_RNA (1)..(19)
acgauaauuucuucuuaacaa

SEQ ID NO: 32 - DNA, 21 bp, Artificial
  siRNA for human TUG1
  misc_RNA (1)..(19)
auuaauaacuaaaaaaucccc

SEQ ID NO: 33 - DNA, 21 bp, Artificial
  siRNA for human TUG1
  misc_RNA (1)..(19)
ugaauuucaaucauuugagat

SEQ ID NO: 34 - DNA, 21 bp, Artificial
  siRNA for human TUG1
  misc_RNA (1)..(19)
uugaaguagaaaaaacagggt

SEQ ID NO: 35 - DNA, 21 bp, Artificial
  siRNA for human TUG1
  misc_RNA (1)..(19)
agaauuucuuacauuugugta

SEQ ID NO: 36 - RNA, 19 nt, Artificial
  LNA-modified antisense RNA
  misc_feature (1)..(4): locked nucleic acid
  misc_feature (16)..(19): locked nucleic acid
uuacucugggcuucugcac

SEQ ID NO: 37 - RNA, 19 nt, Artificial
  LNA-modified antisense RNA
  misc_feature (1)..(3): locked nucleic acid
  misc_feature (17)..(19): locked nucleic acid
uuacucugggcuucugcac

SEQ ID NO: 38 - RNA, 19 nt, Artificial
  LNA-modified antisense RNA
  misc_feature (1)..(4): locked nucleic acid
  misc_feature (17)..(19): locked nucleic acid
uuacucugggcuucugcac

SEQ ID NO: 39 - DNA, 21 bp, Artificial
  siRNA for human TUG1
  misc_RNA (1)..(19)
uacuguuucuuuaaauggcgg

SEQ ID NO: 40 - DNA, 21 bp, Artificial
  siRNA for human TUG1
  misc_RNA (1)..(19)
aaaaguuuagcuuugaaucac

SEQ ID NO: 41 - DNA, 21 bp, Artificial
  siRNA for human TUG1
  misc_RNA (1)..(19)
auaaaugcaucuugauaugtt

SEQ ID NO: 42 - DNA, 21 bp, Artificial
  siRNA for human TUG1
  misc_RNA (1)..(19)
auuaauaacuaaaaaaucccc

SEQ ID NO: 43 - DNA, 19 bp, Artificial
  siRNA for human TUG1
  misc_RNA (1)..(17)
gaauaagcccuauggauta

SEQ ID NO: 44 - DNA, 21 bp, Artificial
  siRNA for human TUG1
  misc_RNA (1)..(19)
uaacuuaagcaaaaaagggta

SEQ ID NO: 45 - DNA, 21 bp, Artificial
  siRNA for human TUG1
  misc_RNA (1)..(19)
gccauuuaaagaaacaguacc

SEQ ID NO: 46 - DNA, 21 bp, Artificial
  siRNA for human TUG1
  misc_RNA (1)..(19)
gauucaaagcuaaacuuuutc

SEQ ID NO: 47 - DNA, 21 bp, Artificial
  siRNA for human TUG1
  misc_RNA (1)..(19)
cauaucaagaugcauuuauta

SEQ ID NO: 48 - DNA, 21 bp, Artificial
  siRNA for human TUG1
  misc_RNA (1)..(19)
ggauuuuuuaguuauuaaugc

SEQ ID NO: 49 - DNA, 19 bp, Artificial
  siRNA for human TUG1
  misc_RNA (1)..(17)
uaauccauagggcuuautc

SEQ ID NO: 50 - DNA, 21 bp, Artificial
  siRNA for human TUG1
  misc_RNA (1)..(19)
cccuuuuuugcuuaaguuact

SEQ ID NO: 51 - RNA, 21 nt, Artificial
  LNA-modified antisense RNA
  misc_feature (1)..(4): locked nucleic acid
  misc_feature (18)..(21): locked nucleic acid
ugaauuucaaucauuugagau

SEQ ID NO: 52 - RNA, 21 nt, Artificial
  LNA-modified antisense RNA
  misc_feature (1)..(3): locked nucleic acid
  misc_feature (19)..(21): locked nucleic acid
ugaauuucaaucauuugagau

SEQ ID NO: 53 - RNA, 21 nt, Artificial
  LNA-modified antisense RNA
  misc_feature (1)..(4): locked nucleic acid
  misc_feature (19)..(21): locked nucleic acid
ugaauuucaaucauuugagau

SEQ ID NO: 54 - DNA, 21 bp, Artificial
  siRNA for firefly GL3 luciferase
  misc_RNA (1)..(19)
cuuacgcugaguacuucgatt

SEQ ID NO: 55 - DNA, 21 bp, Artificial
  siRNA for firefly GL3 luciferase
  misc_RNA (1)..(19)
ucgaaguacucagcguaagtt

SEQ ID NO: 56 - DNA, 21 bp, Artificial
  LNA-modified antisense DNA
  misc_feature (1)..(4): locked nucleic acid
  misc_feature (19)..(21): locked nucleic acid
tgaatttcaatcatttgagat

SEQ ID NO: 57 - DNA, 21 bp, Artificial
  LNA-modified DNA for firefly GL3 luciferase
  misc_feature (1)..(4): locked nucleic acid
  misc_feature (19)..(21): locked nucleic acid
tcgaagtactcagcgtaagtt